European Patent Application EP 4 112 647 A1, published January 4, 2023. Title: ANTI-CD47/ANTI-PD-L1 ANTIBODY AND APPLICATIONS THEREOF. Applicant: NANJING SANHOME PHARMACEUTICAL CO., LTD. The sequence listing filed with the application follows.

SEQUENCE LISTING (134 sequences)

SEQ ID NO: 1 - protein, 8 aa, Artificial sequence
  H1CDR1
GYIFTDYY

SEQ ID NO: 2 - protein, 8 aa, Artificial sequence
  H1CDR2
ITPGSGLT

SEQ ID NO: 3 - protein, 12 aa, Artificial sequence
  H1CDR3
ARCSYGSSFPHV

SEQ ID NO: 4 - protein, 8 aa, Artificial sequence
  VH CDR1 of SHC025-34
GYTFTNYW

SEQ ID NO: 5 - protein, 8 aa, Artificial sequence
  VH CDR2 of SHC025-34
ITPGRGET

SEQ ID NO: 6 - protein, 10 aa, Artificial sequence
  VH CDR3 of SHC025-34
SRWGLRRGDY

SEQ ID NO: 7 - protein, 8 aa, Artificial sequence
  H1CDR1
GFIFSRFG

SEQ ID NO: 8 - protein, 8 aa, Artificial sequence
  H1CDR2
ISSGGSYT

SEQ ID NO: 9 - protein, 14 aa, Artificial sequence
  H1CDR3
ARQGLLDYLYALDY

SEQ ID NO: 10 - protein, 8 aa, Artificial sequence
  H1CDR1
GYTFTDYY

SEQ ID NO: 11 - protein, 12 aa, Artificial sequence
  H1CDR3
ARTSYGSSFPHV

SEQ ID NO: 12 - protein, 12 aa, Artificial sequence
  L1CDR1
QSLLNVNDQKNY

SEQ ID NO: 13 - protein, 3 aa, Artificial sequence
  L1CDR2
FAS

SEQ ID NO: 14 - protein, 9 aa, Artificial sequence
  L1CDR3
QQHYSTPLT

SEQ ID NO: 15 - protein, 7 aa, Artificial sequence
  VL CDR1 of SHC025-34
SSVSSSY

SEQ ID NO: 16 - protein, 3 aa, Artificial sequence
  VL CDR2 of SHC025-34
STS

SEQ ID NO: 17 - protein, 9 aa, Artificial sequence
  VL CDR3 of SHC025-34
QQYSGYPLT

SEQ ID NO: 18 - protein, 6 aa, Artificial sequence
  L1CDR1
QDINSF

SEQ ID NO: 19 - protein, 3 aa, Artificial sequence
  L1CDR2
RAY

SEQ ID NO: 20 - protein, 9 aa, Artificial sequence
  L1CDR3
QQYVEFPPT

SEQ ID NO: 21 - protein, 119 aa, Artificial sequence
  VH of SHC025-26
QVQLKQSGAELVRPGASVKLSCKASGYIFTDYYMNWVKQRPGQGLEWIARIYPGSGLTYYNAKFKGKATVTAEKSSSTAYMQLSSLTSEDSAVYFCARCSYGSSFPHVWGTGTTVTVSS

SEQ ID NO: 22 - protein, 117 aa, Artificial sequence
  VH of SHC025-34
QVQLQQPGAELVKPGASVKMSCKASGYTFTNYWITWVKQRPGQGLEWIGDITPGRGETNYNEKFKSKATLTVDTSSSTAYMQLTSLTSEDSAVYYCSRWGLRRGDYWGQGTSVTVSS

SEQ ID NO: 23 - protein, 121 aa, Artificial sequence
  VH of SHC025-58
EVQLVESGGDLVEPGGSLKLSCAASGFIFSRFGMAWVRQTPDKRLEWVATISSGGSYTYYPDSVKGRLTISRDNAKTTLYLQMRSLKSEDTAMYYCARQGLLDYLYALDYWGQGTAVTVSS

SEQ ID NO: 24 - protein, 113 aa, Artificial sequence
  VL of SHC025-26
DIVMTQSPFSLAMSVGQKVTMSCKSSQSLLNVNDQKNYLAWYQQKPGQSPKLLVYFASTRESGVPDRFIGSGSGTDFTLTISSVQAEDLADYFCQQHYSTPLTFGAGTKLELK

SEQ ID NO: 25 - protein, 108 aa, Artificial sequence
  VL of SHC025-34
ENVLTQSPAIMSASPGEKVTMTCRASSSVSSSYLNWYQQKSGASPKLWIYSTSNLASGVPGRFSGSGSGTSYSLTISSVEAEDAATYYCQQYSGYPLTFGAGTKLEVK

SEQ ID NO: 26 - protein, 107 aa, Artificial sequence
  VL of SHC025-58
DIKMIQSPSSMYAGLGERVTFNCKASQDINSFLCWFQQKPGKSPRPLIYRAYRLVDGVPSRFSGVGSGQDYSLTISSLDYEDLGIYYCQQYVEFPPTFGAGTMLELK

SEQ ID NO: 27 - protein, 119 aa, Artificial sequence
  VH of SHC025-26CHI-T
QVQLKQSGAELVRPGASVKLSCKASGYIFTDYYMNWVKQRPGQGLEWIARIYPGSGLTYYNAKFKGKATVTAEKSSSTAYMQLSSLTSEDSAVYFCARTSYGSSFPHVWGTGTTVTVSS

SEQ ID NO: 28 - protein, 107 aa, Artificial sequence
  VL of SHC025-58CHI-A
DIKMIQSPSSMYAGLGERVTFNCKASQDINSFLAWFQQKPGKSPRPLIYRAYRLVDGVPSRFSGVGSGQDYSLTISSLDYEDLGIYYCQQYVEFPPTFGAGTMLELK

SEQ ID NO: 29 - protein, 119 aa, Artificial sequence
  VH of Hu26T-31-PE
QVQLVQSGAEVKKPGASVKVSCKASGYTFTDYYMNWVRQAPGQGLEWIGRIYPGSGLTYYNAKFKGRATVTADKSTSTVYMELSSLRSEDTAVYYCARTSYGSSFPHVWGQGTTVTVSS

SEQ ID NO: 30 - protein, 117 aa, Artificial sequence
  VH of Hu34-39-PE
QVQLQESGPGLVKPSQTLSLTCKASGYTFTNYWITWVKQRPGQGLEWIGDITPGRGETNYNQKFKGRVTLTVDISASTAYMELSSLRSEDTAVYYCSRWGLRRGDYWGQGTSVTVSS

SEQ ID NO: 31 - protein, 121 aa, Artificial sequence
  VH of Hu58A-14-PE
EVQLLESGGGLVQPGGSLRLSCAASGFIFSRFGMAWVRQTPDKRLEWVATISSGGSYTYYPDSVKGRLTISRDNAKTTLYLQMRSLKSEDTAMYYCARQGLLDYLYALDYWGQGTAVTVSS

SEQ ID NO: 32 - protein, 113 aa, Artificial sequence
  VL of Hu26T-31-PE
DIQMTQSPSSLSASVGDRVTITCKSSQSLLNVNDQKNYLAWYQQKPGKAPKLLIYFASTRESGVPSRFSGSGSGTDFTLTISSLQPEDFATYYCQQHYSTPLTFGQGTKLEIK

SEQ ID NO: 33 - protein, 108 aa, Artificial sequence
  VL of Hu34-39-PE
EIVLTQSPGTLSLSPGERATLSCRASSSVSSSYLNWYQQKSGASPKLWIYSTSNLASGVPGRFSGSGSGTSYSLTISSVEAEDAATYYCQQYSGYPLTFGAGTKLEVK

SEQ ID NO: 34 - protein, 107 aa, Artificial sequence
  VL of Hu58A-14-PE
DIQMTQSPSSVSASIGDRVTITCKASQDINSFLAWFQQKPGKSPRPLIYRAYRLVDGVPSRFSGVGSGQDYSLTISSLDYEDLGIYYCQQYVEFPPTFGAGTMLELK

SEQ ID NO: 35 - DNA, 357 bp, Artificial sequence
  Nucleotide sequence of VH of Hu26T-31-PE
caggtgcagctggtgcagagcggagccgaagtgaagaagcccggtgccagcgtgaaagtaagctgcaaggccagcggctacaccttcaccgactactacatgaactgggtgaggcaggcccctggacaaggcctggagtggatcggcaggatctaccccggcagcggcctgacctactataacgccaagttcaagggcagggccaccgtgaccgccgacaagtccaccagcaccgtgtacatggagctgagcagcctgaggagcgaggacaccgccgtgtattactgcgccaggaccagctacggcagcagcttcccccacgtgtggggccagggcaccaccgtgaccgtgagctct

SEQ ID NO: 36 - DNA, 351 bp, Artificial sequence
  Nucleotide sequence of VH of Hu34-39-PE
caggttcagctgcaagagagcggtcccggcctggtgaaacccagccagaccctgagcctgacctgcaaggccagcggctacactttcactaactactggatcacctgggtgaagcagcgacccggccagggcctggagtggatcggcgacatcacccctgggaggggagagaccaactacaaccagaagttcaagggcagggtgaccctgaccgtggacatcagcgcctccactgcctatatggagctgagcagcctgaggagcgaggacaccgccgtgtactactgcagcaggtggggcctgaggaggggcgattactggggccaagggaccagcgtgaccgtgagctct

SEQ ID NO: 37 - DNA, 363 bp, Artificial sequence
  Nucleotide sequence of VH of Hu58A-14-PE
gaggtccagctgctggagagcggcggtggcctcgtgcagcccggaggcagcctgaggctgagctgcgcggcaagcggcttcatcttcagcaggttcggcatggcctgggtgaggcagaccccagacaagaggctggagtgggtggcaactatcagcagcggaggaagttacacctactaccccgacagcgtgaagggcaggctgaccatcagtagggacaacgccaagaccaccctgtacctgcagatgaggagcctgaagagcgaggacaccgccatgtactactgcgccaggcagggcctgctcgactatctgtacgccctggactattggggccagggcactgccgtgaccgtgagcagc

SEQ ID NO: 38 - DNA, 339 bp, Artificial sequence
  Nucleotide sequence of VL of Hu26T-31-PE
gacatccagatgacccagagcccaagcagcctgagcgccagcgtgggcgacagggtgaccatcacctgcaagagcagccaaagcctgctgaacgtgaacgaccagaagaactacctggcctggtatcagcagaagccgggcaaggcccccaagctgctcatctactttgccagcaccagggagagcggcgtgcccagcaggttcagcggcagcggaagtggcaccgacttcaccctcaccatcagctccctgcaacccgaggacttcgccacctactactgtcaacagcactacagcacacccctgaccttcggccagggcaccaagttggagatcaag

SEQ ID NO: 39 - DNA, 324 bp, Artificial sequence
  Nucleotide sequence of VL of Hu34-39-PE
gagatcgtgctgacccagagccctggcaccttgagcctgagtcccggagagagggccaccctgagctgcagggcctcaagctccgtgagcagcagctatctgaattggtatcagcagaagagcggagccagccccaagctgtggatctacagcaccagcaacctggcaagcggcgtgcccggcaggttcagcggcagtggcagcgggaccagctacagcctgaccatcagtagcgtggaggccgaggacgccgccacctactactgccagcagtacagcggataccctctgaccttcggagccggaaccaagttggaggtgaag

SEQ ID NO: 40 - DNA, 321 bp, Artificial sequence
  Nucleotide sequence of VL of Hu58A-14-PE
gacatccagatgacccagagcccaagcagcgtgagcgccagcatcggcgacagggtgaccataacctgcaaggccagccaagacatcaacagcttcctggcatggttccagcagaagcccggcaagagccccaggcccctgatctacagggcctacaggctggtagacggggtgcccagcaggttcagcggcgtgggcagcggccaggactacagcctgaccatcagcagcctggactacgaggacctgggcatctactactgccagcagtacgtggagttccccccgaccttcggtgcagggaccatgctggagctgaag

SEQ ID NO: 41 - protein, 323 aa, Artificial sequence
  Amino acid sequence of CD47
MWPLVAALLLGSACCGSAQLLFNKTKSVEFTFCNDTVVIPCFVTNMEAQNTTEVYVKWKFKGRDIYTFDGALNKSTVPTDFSSAKIEVSQLLKGDASLKMDKSDAVSHTGNYTCEVTELTREGETIIELKYRVVSWFSPNENILIVIFPIFAILLFWGQFGIKTLKYRSGGMDEKTIALLVAGLVITVIVIVGAILFVPGEYSLKNATGLGLIVTSTGILILLHYYVFSTAIGLTSFVIAILVIQVIAYILAVVGLSLCIAACIPMHGPLLISGLSILALAQLLGLVYMKFVASNQKTIQPPRKAVEEPLNAFKESKGMMNDE

SEQ ID NO: 42 - protein, 350 aa, Artificial sequence
  CD47-Fc fusion protein
QLLFNKTKSVEFTFCNDTVVIPCFVTNMEAQNTTEVYVKWKFKGRDIYTFDGALNKSTVPTDFSSAKIEVSQLLKGDASLKMDKSDAVSHTGNYTCEVTELTREGETIIELKYRVVSWEPKSCDKTHTCPPCPAPELLGGPSVFLFPPKPKDTLMISRTPEVTCVVVDVSHEDPEVKFNWYVDGVEVHNAKTKPREEQYNSTYRVVSVLTVLHQDWLNGKEYKCKVSNKALPAPIEKTISKAKGQPREPQVYTLPPSRDELTKNQVSLTCLVKGFYPSDIAVEWESNGQPENNYKTTPPVLDSDGSFFLYSKLTVDKSRWQQGNVFSCSVMHEALHNHYTQKSLSLSPGK

SEQ ID NO: 43 - protein, 124 aa, Artificial sequence
  CD47-his fusion protein
QLLFNKTKSVEFTFCNDTVVIPCFVTNMEAQNTTEVYVKWKFKGRDIYTFDGALNKSTVPTDFSSAKIEVSQLLKGDASLKMDKSDAVSHTGNYTCEVTELTREGETIIELKYRVVSWHHHHHH

SEQ ID NO: 44 - protein, 354 aa, Artificial sequence
  CD47 extracellular region fusion protein
QLLFNKTKSVEFTFCNDTVVIPCFVTNMEAQNTTEVYVKWKFKGRDIYTFDGALNKSTVPTDFSSAKIEVSQLLKGDASLKMDKSDAVSHTGNYTCEVTELTREGETIIELKYRVVSWFSPEPRGPTIKPCPPCKCPAPNLLGGPSVFIFPPKIKDVLMISLSPIVTCVVVDVSEDDPDVQISWFVNNVEVHTAQTQTHREDYNSTLRVVSALPIQHQDWMSGKEFKCKVNNKDLPAPIERTISKPKGSVRAPQVYVLPPPEEEMTKKQVTLTCMVTDFMPEDIYVEWTNNGKTELNYKNTEPVLDSDGSYFMYSKLRVEKKNWVERNSYSCSVVHEGLHNHHTTKSFSRTPGK

SEQ ID NO: 45 - protein, 338 aa, Artificial sequence
  Amino acid sequence of SIRP
ELQVIQPDKSVLVAAGETATLRCTATSLIPVGPIQWFRGAGPGRELIYNQKEGHFPRVTTVSDLTKRNNMDFSIRIGNITPADAGTYYCVKFRKGSPDDVEFKSGAGTELSVRAKPSAPVVSGPAARATPQHTVSFTCESHGFSPRDITLKWFKNGNELSDFQTNVDPVGESVSYSIHSTAKVVLTREDVHSQVICEVAHVTLQGDPLRGTANLSETIRVPPTLEVTQQPVRAENQVNVTCQVRKFYPQRLQLTWLENGNVSRTETASTVTENKDGTYNWMSWLLVNVSAHRDDVKLTCQVEHDGQPAVSKSHDLKVSAHPKEQGSNTAAENTGSNER

SEQ ID NO: 46 - protein, 466 aa, Artificial sequence
  Heavy chain amino acid sequence of AB06.12-4P
MEFGLSWLFLVAILKGVQCQMQLVQSGAEVKKTGSSVKVSCKASGFNIKDYYLHWVRQAPGQALEWMGWIDPDQGDTEYAQKFQDRVTITRDRSMSTAYMELSSLRSEDTAMYYCNAAYGSSSYPMDYWGQGTTVTVSSASTKGPSVFPLAPCSRSTSESTAALGCLVKDYFPEPVTVSWNSGALTSGVHTFPAVLQSSGLYSLSSVVTVPSSSLGTKTYTCNVDHKPSNTKVDKRVESKYGPPCPPCPAPEFLGGPSVFLFPPKPKDTLMISRTPEVTCVVVDVSQEDPEVQFNWYVDGVEVHNAKTKPREEQFNSTYRVVSVLTVLHQDWLNGKEYKCKVSNKGLPSSIEKTISKAKGQPREPQVYTLPPSQEEMTKNQVSLTCLVKGFYPSDIAVEWESNGQPENNYKTTPPVLDSDGSFFLYSRLTVDKSRWQEGNVFSCSVMHEALHNHYTQKSLSLSLGK

SEQ ID NO: 47 - protein, 236 aa, Artificial sequence
  Light chain amino acid sequence of AB06.12-4P
MDMRVPAQLLGLLLLWFPGSRCNIQMTQSPSAMSASVGDRVTITCKASQDIHRYLSWFQQKPGKVPKHLIYRANRLVSGVPSRFSGSGSGTEFTLTISSLQPEDFATYYCLQYDEFPYTFGGGTKVEIKRTVAAPSVFIFPPSDEQLKSGTASVVCLLNNFYPREAKVQWKVDNALQSGNSQESVTEQDSKDSTYSLSSTLTLSKADYEKHKVYACEVTHQGLSSPVTKSFNRGEC

SEQ ID NO: 48 - protein, 117 aa, Artificial sequence
  Humanized VH of SHC025-34CHI
QVQLQESGGGVVQPGRSLRLSCKASGYTFTNYWITWVKQRPGQGLEWIGDITPGRGETNYNPSLKSRLTISIDTSKTQFSLKLSSVTAADTAIYYCSRWGLRRGDYWGQGTSVTVSS

SEQ ID NO: 49 - protein, 117 aa, Artificial sequence
  Humanized VH of SHC025-34CHI
QVQLQQPGAELVKPGASVKMSCKASGYTFTNYWITWVKQRPGQGLEWIGDITPGRGETNYNPSLKSRLTISIDTSKTQFSLKLSSVTAADTAIYYCSRWGLRRGDYWGQGTSVTVSS

SEQ ID NO: 50 - protein, 117 aa, Artificial sequence
  Humanized VH of SHC025-34CHI
QVQLQESGGGVVQPGRSLRLSCKASGYTFTNYWITWVKQRPGQGLEWIGDITPGRGETNYNEKFKSKATLTVDTSSSTAYMQLTSLTSEDSAVYYCSRWGLRRGDYWGQGTSVTVSS

SEQ ID NO: 51 - protein, 118 aa, Artificial sequence
  Humanized VH of SHC025-34CHI
QVQLQESGPGLVRPSQTLSLTCKASGYTFTNYWITWVKQRPGQGLEWIGDITPGRGETNYNPSLKSRLTISIDTSKTQFSLKLSSVTAADTAIYYCSRWGLRRGDYWGQGTSVTVSSH

SEQ ID NO: 52 - protein, 117 aa, Artificial sequence; identical to SEQ ID NO: 30
  Humanized VH of SHC025-34CHI

SEQ ID NO: 53 - protein, 117 aa, Artificial sequence
  Humanized VH of SHC025-34CHI
QVQLQESGGGVVQPGRSLRLSCKASGYTFTNYWITWVKQRPGQGLEWIGDITPGRGETNYNQKFKGRVTLTVDISASTAYMELSSLRSEDTAVYYCSRWGLRRGDYWGQGTSVTVSS

SEQ ID NO: 54 - protein, 108 aa, Artificial sequence
  Humanized VL of SHC025-34CHI
EIVLTQSPATLSLSPGERATLSCRASSSVSSSYLNWYQQKSGASPKLWIYSTSNLASGVPGRFSGSGSGTSYSLTISSVEAEDAATYYCQQYSGYPLTFGAGTKLEVK

SEQ ID NO: 55 - protein, 108 aa, Artificial sequence
  Humanized VL of SHC025-34CHI
EIVLTQSPATLSLSPGERATLSCRASSSVSSSYLNWYQQKSGASPKLWIYSTSNLASGVPSRFSGSGSGTSFTLTISSLQPEDAATYYCQQYSGYPLTFGAGTKLEVK

SEQ ID NO: 56 - protein, 108 aa, Artificial sequence; identical to SEQ ID NO: 33
  Humanized VL of SHC025-34CHI

SEQ ID NO: 57 - protein, 108 aa, Artificial sequence
  Humanized VL of SHC025-34CHI
EIVMTQSPATLSLSPGERATLSCRASSSVSSSYLNWYQQKSGASPKLWIYSTSNLASGVPGRFSGSGSGTSYSLTISSVEAEDAATYYCQQYSGYPLTFGAGTKLEVK

SEQ ID NO: 58 - protein, 121 aa, Artificial sequence
  Humanized VH of SHC025-58CHI-A
EVQLVESGGDLVEPGGSLKLSCAASGFIFSRFGMAWVRQTPDKRLEWVATISSGGSYTRYSPSFQGQVTMSVDKSITTAYLQWNSLKASDTAMYYCARQGLLDYLYALDYWGQGTAVTVSS

SEQ ID NO: 59 - protein, 121 aa, Artificial sequence
  Humanized VH of SHC025-58CHI-A
QVQLVESGGGVVQPGRSLRLSCAASGFIFSRFGMAWVRQTPDKRLEWVATISSGGSYTYYPDSVKGRLTISRDNAKTTLYLQMRSLKSEDTAMYYCARQGLLDYLYALDYWGQGTAVTVSS

SEQ ID NO: 60 - protein, 121 aa, Artificial sequence
  Humanized VH of SHC025-58CHI-A
LVQLVESGGGLIQPGGSLRLSCAASGFIFSRFGMAWVRQTPDKRLEWVATISSGGSYTNYNQKFKGRVTLTVDISASTAYMELSSLRSEDTAVYYCARQGLLDYLYALDYWGQGTAVTVSS

SEQ ID NO: 61 - protein, 121 aa, Artificial sequence; identical to SEQ ID NO: 31
  Humanized VH of SHC025-58CHI-A

SEQ ID NO: 62 - protein, 121 aa, Artificial sequence
  Humanized VH of SHC025-58CHI-A
LVQLVESGGGLIQPGGSLRLSCAASGFIFSRFGMAWVRQTPDKRLEWVATISSGGSYTRYSPSFQGQVTMSVDKSITTAYLQWNSLKASDTAMYYCARQGLLDYLYALDYWGQGTAVTVSS

SEQ ID NO: 63 - protein, 121 aa, Artificial sequence
  Humanized VH of SHC025-58CHI-A
EVQLLESGGGLVQPGGSLRLSCAASGFIFSRFGMAWVRQTPDKRLEWVATISSGGSYTRYSPSFQGQVTMSVDKSITTAYLQWNSLKASDTAMYYCARQGLLDYLYALDYWGQGTAVTVSS

SEQ ID NO: 64 - protein, 107 aa, Artificial sequence
  Humanized VL of SHC025-58CHI-A
DIQMTQSPSSVSASIGDRVTITCKASQDINSFLTWFQQKPGKSPRPLIYRAYRLVDGVPSRFSGVGSGQDYSLTISSLDYEDLGIYYCQQYVEFPPTFGAGTMLELK

SEQ ID NO: 65 - protein, 107 aa, Artificial sequence
  Humanized VL of SHC025-58CHI-A
DIQMTQSPSSVSASIGDRVTITCKASQDINSFLTWFQQKPGKSPRPLIYRAYRLVDGVPSRFSGSGSGTYFTLTISSLQAEDFAVYYCQQYVEFPPTFGAGTMLELK

SEQ ID NO: 66 - protein, 107 aa, Artificial sequence
  Humanized VL of SHC025-58CHI-A
DIKMIQSPSSMYAGLGERVTFNCKASQDINSFLTWFQQKPGKSPRPLIYRAYRLVDGVPSRFSGSGSGTYFTLTISSLQAEDFAVYYCQQYVEFPPTFGAGTMLELK

SEQ ID NO: 67 - protein, 107 aa, Artificial sequence
  Humanized VL of SHC025-58CHI-A
DIQMTQSPSSVSASIGDRVTITCKASQDINSFLTWFQQKPGKSPRPLIYRAYRLVDGVPDRFSGSGSGTDFTLTISSLQAEDVAVYYCQQYVEFPPTFGAGTMLELK

SEQ ID NO: 68 - protein, 107 aa, Artificial sequence
  Humanized VL of SHC025-58CHI-A
DIKMIQSPSSMYAGLGERVTFNCKASQDINSFLTWFQQKPGKSPRPLIYRAYRLVDGVPSRFSGVGSGQDYSLTISSLDYEDLGIYYCQQYVEFPPTFGAGTMLELK

SEQ ID NO: 69 - protein, 119 aa, Artificial sequence
  Humanized VH of SHC025-26CHI-T
QVQLVQSGAEVKKPGASVKVSCKASGYTFTDYYMNWVRQAPGQGLEWMGRIYPGSGLTYYNAKFKGRVTMTRDTSTSTVYMELSSLRSEDTAVYYCARTSYGSSFPHVWGQGTTVTVSS

SEQ ID NO: 70 - protein, 119 aa, Artificial sequence
  Humanized VH of SHC025-26CHI-T
QVQLVQSGAEVKKPGASVKVSCKASGYTFTDYYMNWVRQAPGQGLEWMGRIYPGSGLTYYNAKFKGRVTMTADKSTSTVYMELSSLRSEDTAVYYCARTSYGSSFPHVWGQGTTVTVSS

SEQ ID NO: 71 - protein, 119 aa, Artificial sequence; identical to SEQ ID NO: 29
  Humanized VH of SHC025-26CHI-T

SEQ ID NO: 72 - protein, 119 aa, Artificial sequence
  Humanized VH of SHC025-26CHI-T
QVQLVQSGAEVKKPGASVKVSCKASGYTFTDYYMNWVRQAPGQGLEWIGRIYPGSGLTYYNAKFKGRATVTADKSTSTVYMELSSLRSEDTAVYFCARTSYGSSFPHVWGQGTTVTVSS

SEQ ID NO: 73 - protein, 113 aa, Artificial sequence; identical to SEQ ID NO: 32
  Humanized VL of SHC025-26CHI-T

SEQ ID NO: 74 - protein, 113 aa, Artificial sequence
  Humanized VL of SHC025-26CHI-T
DIQMTQSPSSLSASVGDRVTITCKSSQSLLNVNDQKNYLAWYQQKPGKAPKLLVYFASTRESGVPSRFSGSGSGTDFTLTISSLQPEDFATYFCQQHYSTPLTFGQGTKLEIK

SEQ ID NO: 75 - protein, 10 aa, Artificial sequence
  H2CDR1
GDSITSGYWN

SEQ ID NO: 76 - protein, 16 aa, Artificial sequence
  H2CDR2
YISYTGSTYYNLSLKS

SEQ ID NO: 77 - protein, 10 aa, Artificial sequence
  H2CDR3
YILWLRHFDY

SEQ ID NO: 78 - protein, 17 aa, Artificial sequence
  L2CDR1
KSSQSLLYSSNQKNSLA

SEQ ID NO: 79 - protein, 7 aa, Artificial sequence
  L2CDR2
WASTRES

SEQ ID NO: 80 - protein, 9 aa, Artificial sequence
  L2CDR3
QQYYGYPLT

SEQ ID NO: 81 - protein, 5 aa, Artificial sequence
  H2CDR1
SDYWN

SEQ ID NO: 82 - protein, 16 aa, Artificial sequence
  H2CDR2
YISYTGSTYYNPSLKR

SEQ ID NO: 83 - protein, 10 aa, Artificial sequence
  H2CDR3
YRDWPGYFDV

SEQ ID NO: 84 - protein, 11 aa, Artificial sequence
  L2CDR1
RASKSIRKFLA

SEQ ID NO: 85 - protein, 7 aa, Artificial sequence
  L2CDR2
SGSTLQS

SEQ ID NO: 86 - protein, 9 aa, Artificial sequence
  L2CDR3
QHYNEYPFT

SEQ ID NO: 87 - protein, 10 aa, Artificial sequence
  H2CDR1
GYTFTRNTMH

SEQ ID NO: 88 - protein, 17 aa, Artificial sequence
  H2CDR2
FIDPHNTYTRYNQKFKD

SEQ ID NO: 89 - protein, 5 aa, Artificial sequence
  H2CDR3
WPMDY

SEQ ID NO: 90 - protein, 17 aa, Artificial sequence
  L2CDR1
KSSQSLSWSENQNNYLS

SEQ ID NO: 91 - protein, 7 aa, Artificial sequence
  L2CDR2
GASIRES

SEQ ID NO: 92 - protein, 11 aa, Artificial sequence
  L2CDR3
QHNHGSFLPYT

SEQ ID NO: 93 - protein, 5 aa, Artificial sequence
  H2CDR1
SNWMN

SEQ ID NO: 94 - protein, 17 aa, Artificial sequence
  H2CDR2
MIHLYDSETKLNPNFQD

SEQ ID NO: 95 - protein, 9 aa, Artificial sequence
  H2CDR3
SAGNYRFAY

SEQ ID NO: 96 - protein, 11 aa, Artificial sequence
  L2CDR1
KASQSVSNEVA

SEQ ID NO: 97 - protein, 7 aa, Artificial sequence
  L2CDR2
SASSRYT

SEQ ID NO: 98 - protein, 9 aa, Artificial sequence
  L2CDR3
QQHYSSPLT

SEQ ID NO: 99 - protein, 118 aa, Artificial sequence
  VH of anti-PD-L1
EVQLQESGPSLVKPSQTLSLTCSVTGDSITSGYWNWIRKFPGNKLEYMGYISYTGSTYYNLSLKSRISITRDTSKNQYYLQLNSVTTEDTATYYCARYILWLRHFDYWGQGTTLTVSS

SEQ ID NO: 100 - protein, 118 aa, Artificial sequence
  VH of anti-PD-L1
EVQLQESGPGLAKPSQTLSLTCSVTGYSITSDYWNWIRKFPGNKLEYMGYISYTGSTYYNPSLKRRVSITRDTSKNNYYLQLNSVTTEDTATYYCARYRDWPGYFDVWGAGTTVTVSS

SEQ ID NO: 101 - protein, 114 aa, Artificial sequence
  VH of anti-PD-L1
QVQLQQSGAELARPGASVKMSCKASGYTFTRNTMHWIKQRPGQGLEWIGFIDPHNTYTRYNQKFKDRATLTADKSSSTAYMQLSSLSSEDSAVYYCARWPMDYWGQGTSVTVSS

SEQ ID NO: 102 - protein, 118 aa, Artificial sequence
  VH of anti-PD-L1
QVQLQQPGAELVRPGTSVNLSCKASGYSFTSNWMNWVKQRPGQGLEWIGMIHLYDSETKLNPNFQDKATLTVDKSSSIAYMQLSSPTSEDSAVYYCARSAGNYRFAYWGQGTLVTVSA

SEQ ID NO: 103 - protein, 113 aa, Artificial sequence
  VL of anti-PD-L1
DIVMSQSPSSLAVSVGEKVTMSCKSSQSLLYSSNQKNSLAWYQQKPGQSPKLLIYWASTRESGVPDRFTGSGSGTDFTLTISSVKAEDLAVYYCQQYYGYPLTFGAGTKLELK

SEQ ID NO: 104 - protein, 107 aa, Artificial sequence
  VL of anti-PD-L1
DVQITQSPSYLAASPGETITINCRASKSIRKFLAWYQEKPGKTNKLLIYSGSTLQSGIPSRFSGSGSGTDFTLTISTLEPEDFAVYYCQHYNEYPFTFGGGTKLEIK

SEQ ID NO: 105 - protein, 115 aa, Artificial sequence
  VL of anti-PD-L1
DIVMTQFPSSLAVTAGEKVTMRCKSSQSLSWSENQNNYLSWYQQKQGQPPKLLIYGASIRESWVPDRFTGSGSGTDFTLTISNVHAEDLGVYFCQHNHGSFLPYTFGGGTKLEIK

SEQ ID NO: 106 - protein, 107 aa, Artificial sequence
  VL of anti-PD-L1
SIVMTQTPKFLPVTAEDRVTITCKASQSVSNEVAWYQQKPGQSPKLLIYSASSRYTGVPDRFIGGGSATDFTFTISSVQVEDLAVYFCQQHYSSPLTFGAGTKLELK

SEQ ID NO: 107 - protein, 99 aa, Artificial sequence
  Human antibody germline gene M99683 IGHV4-31x02
QVQLQESGPGLVKPSQTLSLTCTVSGGSISSGGYYWSWIRQHPGKGLEWIGYIYYSGSTYYNPSLKSRVTISVDTSKNQFSLKLSSVTAADTAVYYCAR

SEQ ID NO: 108 - protein, 98 aa, Artificial sequence
  Human antibody germline gene X62109 IGHV1-3x01
QVQLVQSGAEVKKPGASVKVSCKASGYTFTSYAMHWVRQAPGQRLEWMGWINAGNGNTKYSQKFQGRVTITRDTSASTAYMELSSLRSEDTAVYYCAR

SEQ ID NO: 109 - protein, 101 aa, Artificial sequence
  Human antibody germline gene Z00023 IGKV4-1x01
DIVMTQSPDSLAVSLGERATINCKSSQSVLYSSNNKNYLAWYQQKPGQPPKLLIYWASTRESGVPDRFSGSGSGTDFTLTISSLQAEDVAVYYCQQYYSTP

SEQ ID NO: 110 - protein, 118 aa, Artificial sequence
  VH of anti-PD-L1
QVQLQESGPGLVKPSQTLSLTCTVSGDSITSGYWNWIRQHPGKGLEWIGYISYTGSTYYNLSLKSRVTISVDTSKNQFSLKLSSVTAADTAVYYCARYILWLRHFDYWGQGTLVTVSS

SEQ ID NO: 111 - protein, 118 aa, Artificial sequence
  VH of anti-PD-L1
QVQLQESGPGLVKPSQTLSLTCTVSGDSITSGYWNWIRQHPGKGLEYIGYISYTGSTYYNLSLKSRVTISVDTSKNQFSLKLSSVTAADTAVYYCARYILWLRHFDYWGQGTLVTVSS

SEQ ID NO: 112 - protein, 118 aa, Artificial sequence
  VH of anti-PD-L1
QVQLQESGPGLVKPSQTLSLTCTVSGDSITSGYWNWIRQHPGKGLEYIGYISYTGSTYYNLSLKSRVTISRDTSKNQFSLKLSSVTAADTAVYYCARYILWLRHFDYWGQGTLVTVSS

SEQ ID NO: 113 - protein, 118 aa, Artificial sequence
  VH of anti-PD-L1
QVQLQESGPGLVKPSQTLSLTCTVSGDSITSGYWNWIRQHPGKGLEYIGYISYTGSTYYNLSLKSRITISRDTSKNQYSLKLSSVTAADTAVYYCARYILWLRHFDYWGQGTLVTVSS

SEQ ID NO: 114 - protein, 118 aa, Artificial sequence
  VH of anti-PD-L1
QVQLQESGPGLVKPSQTLSLTCTVSGDSITSGYWNWIRQHPGKGLEYMGYISYTGSTYYNLSLKSRITISRDTSKNQYSLKLSSVTAADTAVYYCARYILWLRHFDYWGQGTLLTVSS

SEQ ID NO: 115 - protein, 113 aa, Artificial sequence
  VL of anti-PD-L1
DIVMTQSPDSLAVSLGERATINCKSSQSLLYSSNQKNSLAWYQQKPGQPPKLLIYWASTRESGVPDRFSGSGSGTDFTLTISSLQAEDVAVYYCQQYYGYPLTFGGGTKLEIK

SEQ ID NO: 116 - protein, 113 aa, Artificial sequence
  VL of anti-PD-L1
DIVMTQSPDSLAVSLGERATISCKSSQSLLYSSNQKNSLAWYQQKPGQPPKLLIYWASTRESGVPDRFSGSGSGTDFTLTISSLQAEDVAVYYCQQYYGYPLTFGGGTKLEIK

SEQ ID NO: 117 - protein, 113 aa, Artificial sequence
  VL of anti-PD-L1
DIVMTQSPDSLAVSLGERVTISCKSSQSLLYSSNQKNSLAWYQQKPGQPPKLLIYWASTRESGVPDRFSGSGSGTDFTLTISSVQAEDVAVYYCQQYYGYPLTFGGGTKLEIK

SEQ ID NO: 118 - protein, 113 aa, Artificial sequence
  VL of anti-PD-L1
DIVMTQSPDSLAVSLGERVTMSCKSSQSLLYSSNQKNSLAWYQQKPGQPPKLLIYWASTRESGVPDRFSGSGSGTDFTLTISSVQAEDVAVYYCQQYYGYPLTFGGGTKLEIK

SEQ ID NO: 119 - protein, 114 aa, Artificial sequence
  VH of anti-PD-L1
QVQLVQSGAEVKKPGASVKVSCKASGYTFTRNTMHWVRQAPGQRLEWMGFIDPHNTYTRYNQKFKDRVTITRDTSASTAYMELSSLRSEDTAVYYCARWPMDYWGQGTLVTVSS

SEQ ID NO: 120 - protein, 114 aa, Artificial sequence
  VH of anti-PD-L1
QVQLVQSGAEVKKPGASVKVSCKASGYTFTRNTMHWVRQAPGQRLEWMGFIDPHNTYTRYNQKFKDRVTITADTSASTAYMELSSLRSEDTAVYYCARWPMDYWGQGTLVTVSS

SEQ ID NO: 121 - protein, 114 aa, Artificial sequence
  VH of anti-PD-L1
QVQLVQSGAEVKKPGASVKVSCKASGYTFTRNTMHWIRQAPGQRLEWMGFIDPHNTYTRYNQKFKDRVTITADTSASTAYMELSSLRSEDTAVYYCARWPMDYWGQGTLVTVSS

SEQ ID NO: 122 - protein, 114 aa, Artificial sequence
  VH of anti-PD-L1
QVQLVQSGAEVAKPGASVKVSCKASGYTFTRNTMHWIRQAPGQRLEWIGFIDPHNTYTRYNQKFKDRATITADTSASTAYMELSSLRSEDTAVYYCARWPMDYWGQGTLVTVSS

SEQ ID NO: 123 - protein, 114 aa, Artificial sequence
  VH of anti-PD-L1
QVQLVQSGAEVAKPGASVKMSCKASGYTFTRNTMHWIKQAPGQRLEWIGFIDPHNTYTRYNQKFKDRATLTADTSASTAYMELSSLRSEDTAVYYCARWPMDYWGQGTLVTVSS

SEQ ID NO: 124 - protein, 115 aa, Artificial sequence
  VL of anti-PD-L1
DIVMTQSPDSLAVSLGERATINCKSSQSLSWSENQNNYLSWYQQKPGQPPKLLIYGASIRESGVPDRFSGSGSGTDFTLTISSLQAEDVAVYYCQHNHGSFLPYTFGQGTKLEIK

SEQ ID NO: 125 - protein, 115 aa, Artificial sequence
  VL of anti-PD-L1
DIVMTQSPDSLAVSLGERVTINCKSSQSLSWSENQNNYLSWYQQKPGQPPKLLIYGASIRESGVPDRFSGSGSGTDFTLTISSVQAEDVGVYYCQHNHGSFLPYTFGQGTKLEIK

SEQ ID NO: 126 - protein, 115 aa, Artificial sequence
  VL of anti-PD-L1
DIVMTQSPDSLAVSLGERVTMRCKSSQSLSWSENQNNYLSWYQQKPGQPPKLLIYGASIRESGVPDRFSGSGSGTDFTLTISSVQAEDVGVYYCQHNHGSFLPYTFGQGTKLEIK

SEQ ID NO: 127 - DNA, 354 bp, Artificial sequence
  Nucleotide sequence encoding VH of anti-PD-L1
caggttcagctgcaggagtccggccctggcctggtgaagcccagccagaccctgagcctgacctgtaccgtgagcggcgacagcatcactagcggctactggaactggatcaggcaacaccccggcaagggcctggagtacatcggctacatcagctacaccggcagcacctactacaacctgagtctgaagagcagggtgaccatcagccgggacaccagcaagaaccagttctctctgaagctgagcagcgtgactgcggcggataccgccgtgtactactgcgccaggtacatcctgtggttgaggcacttcgactactggggccagggcaccctggtgaccgttagctct

SEQ ID NO: 128 - DNA, 342 bp, Artificial sequence
  Nucleotide sequence encoding VH of anti-PD-L1
caggtgcagctggtgcagagcggagctgaggtggccaagccaggcgccagcgtgaagatgtcctgcaaggccagcggctacacctttacccggaacacaatgcactggattaagcaggcccccggccagcggctggagtggatcggcttcatcgacccacacaatacctacaccagatacaaccagaagtttaaggaccgggccaccctgaccgccgatacatcagcatcaacagcttacatggagctgagtagtctgagatctgaggatacagccgtgtactattgcgctagatggcctatggattactggggccagggaaccctggtgaccgtgtctagc

SEQ ID NO: 129 - DNA, 339 bp, Artificial sequence
  Nucleotide sequence encoding VL of anti-PD-L1
gacatcgtgatgacccagagccccgactccctggccgtgagcctgggcgagagggccaccatctcctgcaagagcagtcagagccttctgtatagctccaaccagaagaacagcctggcctggtatcaacagaagcccggtcaaccccccaagctgctgatctactgggcctcaaccagggaaagcggcgtgcccgacaggttcagcggcagtggcagcggcaccgacttcaccctgaccatcagctccttgcaggccgaggacgtggcagtgtactactgccagcagtactacggctaccccctgacattcggagggggaaccaagttggagatcaag

SEQ ID NO: 130 - DNA, 345 bp, Artificial sequence
  Nucleotide sequence encoding VL of anti-PD-L1
gatatcgtgatgacccagagcccagatagcctggccgtgagcctgggagagagagtgaccatgagatgtaagtctagtcagagtctgagttggagcgagaatcagaacaattacctgagctggtatcagcagaagcctggccagcctccaaagctgctgatctacggcgcctccatccgggagagcggagtgcccgaccgcttcagcggcagcggcagcggcacagacttcaccctgaccatcagcagcgtgcaggccgaggatgtgggcgtgtactactgtcagcacaaccacggcagcttcctgccctacaccttcgggcagggcaccaagctggagatcaag

SEQ ID NO: 131 - protein, 107 aa, Artificial sequence [sequence omitted]

SEQ ID NO: 132 - protein, 327 aa, Artificial sequence
  IgG4 heavy chain constant region
ASTKGPSVFPLAPCSRSTSESTAALGCLVKDYFPEPVTVSWNSGALTSGVHTFPAVLQSSGLYSLSSVVTVPSSSLGTKTYTCNVDHKPSNTKVDKRVESKYGPPCPPCPAPEFEGGPSVFLFPPKPKDTLMISRTPEVTCVVVDVSQEDPEVQFNWYVDGVEVHNAKTKPREEQFNSTYRVVSVLTVLHQDWLNGKEYKCKVSNKGLPSSIEKTISKAKGQPREPQVYTLPPCQEEMTKNQVSLWCLVKGFYPSDIAVEWESNGQPENNYKTTPPVLDSDGSFFLYSRLTVDKSRWQEGNVFSCSVMHEALHNHYTQKSLSLSLGK

SEQ ID NO: 133 - protein, 327 aa, Artificial sequence
  IgG4 heavy chain constant region
ASTKGPSVFPLAPCSRSTSESTAALGCLVKDYFPEPVTVSWNSGALTSGVHTFPAVLQSSGLYSLSSVVTVPSSSLGTKTYTCNVDHKPSNTKVDKRVESKYGPPCPPCPAPEFEGGPSVFLFPPKPKDTLMISRTPEVTCVVVDVSQEDPEVQFNWYVDGVEVHNAKTKPREEQFNSTYRVVSVLTVLHQDWLNGKEYKCKVSNKGLPSSIEKTISKAKGQPREPQVCTLPPSQEEMTKNQVSLSCAVKGFYPSDIAVEWESNGQPENNYKTTPPVLDSDGSFFLVSRLTVDKSRWQEGNVFSCSVMHEALHNHYTQKSLSLSLGK

SEQ ID NO: 134 - protein, 220 aa, Artificial sequence
  Human PD-L1 extracellular region
FTVTVPKDLYVVEYGSNMTIECKFPVEKQLDLAALIVYWEMEDKNIIQFVHGEEDLKVQHSSYRQRARLLKDQLSLGNAALQITDVKLQDAGVYRCMISYGGADYKRITVKVNAPYNKINQRILVVDPVTSEHELTCQAEGYPKAEVIWTSSDHQVLSGKTTTTNSKREEKLFNVTSTLRINTTTNEIFYCTFRRLDPEENHTAELVIPELPLAHPPNER